European Patent Application EP 4 793 351 A1, published August 19, 2026. Title: 载体对与宿主细胞和高表达细胞株的构建方法. Applicant: 上海药明生物技术有限公司. Application CN. The sequence listing filed with the application follows.

SEQUENCE LISTING (13 sequences)

SEQ ID NO: 1 - protein, 124 aa, Streptoalloteichus hindustanus
MAKLTSAVPVLTARDVAGAVEFWTDRLGFSRDFVEDDFAGVVRDDVTLFISAVQDQVVPDNTLAWVWVRGLDELYAEWSEVVSTNFRDASGPAMTEIGEQPWGREFALRDPAGNCVHFVAEEQD

SEQ ID NO: 2 - protein, 94 aa, synthetic construct
MAKLTSAVPVLTARDVAGAVEFWTDRLGFSRDFVEDDFAGVVRDDVTLFISAVQDQVVPDNGSGGALKKELQANKKELAQLKWELQALKKELAQ

SEQ ID NO: 3 - protein, 98 aa, synthetic construct
MEQLEKKLQALEKKLAQLEWKNQALEKKLAQGSGGTLAWVWVRGLDELYAEWSEVVSTNFRDASGPAMTEIGEQPWGREFALRDPAGNCVHFVAEEQD

SEQ ID NO: 4 - protein, 94 aa, synthetic construct
MAKLTSAVPVLTARDVAEAVEFWTDRLGFSRVFVEDDFAGVVRDDVTLFISAVQDQVVPDNGSGGALKKELQANKKELAQLKWELQALKKELAQ

SEQ ID NO: 5 - protein, 98 aa, synthetic construct
MEQLEKKLQALEKKLAQLEWKNQALEKKLAQGSGGTQAWVWVRGLDELYAEWSEVVSTNFRDASGPAMTEIVEQPWGREFALRDPAGNCVHFVAEEQD

SEQ ID NO: 6 - protein, 98 aa, synthetic construct
MEQLEKKLQALEKKLAQLEWKNQALEKKLAQGGGGGSAKLTSAVPVLTARDVAGAVEFWTDRLGFSRDFVEDDFAGVVRDDVTLFISAVQDQVVPDNT

SEQ ID NO: 7 - protein, 95 aa, synthetic construct
MLAWVWVRGLDELYAEWSEVVSTNFRDASGPAMTEIGEQPWGREFALRDPAGNCVHFVAEGGGGGGALKKELQANKKELAQLKWELQALKKELAQ

SEQ ID NO: 8 - protein, 98 aa, synthetic construct
MEQLEKKLQALEKKLAQLEWKNQALEKKLAQGGGGGSAKLTSAVPVLTARDVAEAVEFWTDRLGFSRVFVEDDFAGVVRDDVTLFISAVQDQVVPDNT

SEQ ID NO: 9 - protein, 95 aa, synthetic construct
MQAWVWVRGLDELYAEWSEVVSTNFRDASGPAMTEIVEQPWGREFALRDPAGNCVHFVAEGGGGGGALKKELQANKKELAQLKWELQALKKELAQ

SEQ ID NO: 10 - protein, 30 aa, synthetic construct
EQLEKKLQALEKKLAQLEWKNQALEKKLAQ

SEQ ID NO: 11 - protein, 29 aa, synthetic construct
ALKKELQANKKELAQLKWELQALKKELAQ

SEQ ID NO: 12 - protein, 451 aa, synthetic construct
EVQLVESGGGLVQPGRSLRLSCAASGFTFDDYAMHWVRQAPGKGLEWVSAITWNSGHIDYADSVEGRFTISRDNAKNSLYLQMNSLRAEDTAVYYCAKVSYLSTASSLDYWGQGTLVTVSSASTKGPSVFPLAPSSKSTSGGTAALGCLVKDYFPEPVTVSWNSGALTSGVHTFPAVLQSSGLYSLSSVVTVPSSSLGTQTYICNVNHKPSNTKVDKKVEPKSCDKTHTCPPCPAPELLGGPSVFLFPPKPKDTLMISRTPEVTCVVVDVSHEDPEVKFNWYVDGVEVHNAKTKPREEQYNSTYRVVSVLTVLHQDWLNGKEYKCKVSNKALPAPIEKTISKAKGQPREPQVYTLPPSRDELTKNQVSLTCLVKGFYPSDIAVEWESNGQPENNYKTTPPVLDSDGSFFLYSKLTVDKSRWQQGNVFSCSVMHEALHNHYTQKSLSLSPGK

SEQ ID NO: 13 - protein, 214 aa, synthetic construct
DIQMTQSPSSLSASVGDRVTITCRASQGIRNYLAWYQQKPGKAPKLLIYAASTLQSGVPSRFSGSGSGTDFTLTISSLQPEDVATYYCQRYNRAPYTFGQGTKVEIKRTVAAPSVFIFPPSDEQLKSGTASVVCLLNNFYPREAKVQWKVDNALQSGNSQESVTEQDSKDSTYSLSSTLTLSKADYEKHKVYACEVTHQGLSSPVTKSFNRGEC